European Patent Application EP 4 733 319 A1, published April 29, 2026. Title: THERAPEUTIC MOLECULES. Applicant: Kyron.bio. Application EP. The sequence listing filed with the application follows.

SEQUENCE LISTING (6 sequences)

SEQ ID NO: 1 - protein, 451 aa, synthetic construct
EVQLVESGGGLVQPGRSLRLSCAASGFTFDDYAMHWVRQAPGKGLEWVSAITWNSGHIDYADSVEGRFTISRDNAKNSLYLDMNSLRAEDTAVYYCAKVSYLSTASSLDYWGQGTLVTVSSASTKGPSVFPLAPSSKSTSGGTAALGCLVKDYFPEPVTVSWNSGALTSGVHTFPAVLQSSGLYSLSSVVTVPSSSLGTQTYICNVNHKPSNTKVDKKVEPKSCDKTHTCPPCPAPELLGGPSVFLFPPKPKDTLMISRTPEVTCVVVDVSHEDPEVKFNWYVDGVEVHNAKTKPREEQYNSTYRVVSVLTVLHQDWLNGKEYKCKVSNKALPAPIEKTISKAKGQPREPQVYTLPPSRDELTKNQVSLTCLVKGFYPSDIAVEWESNGQPENNYKTTPPVLDSDGSFFLYSKLTVDKSRWQQGNVFSCSVMHEALHNHYTQKSLSLSPGK

SEQ ID NO: 2 - protein, 214 aa, synthetic construct
DIQMTQSPSSLSASVGDRVTITCRASQGIRNYLAWYQQKPGKAPKLLIYAASTLQSGVPSRFSGSGSGTDFTLTISSLQPEDVATYYCQRYNRAPYTFGQGTKVEIKRTVAAPSVFIFPPSDEQLKSGTASVVCLLNNFYPREAKVQWKVDNALQSGNSQESVTEQDSKDSTYSLSSTLTLSKADYEKHKVYACEVTHQGLSSPVTKSFNRGEC

SEQ ID NO: 3 - protein, 121 aa, synthetic construct
EVQLVESGGGLVQPGRSLRLSCAASGFTFDDYAMHWVRQAPGKGLEWVSAITWNSGHIDYADSVEGRFTISRDNAKNSLYLDMNSLRAEDTAVYYCAKVSYNSTASSLDYWGQGTLVTVSS

SEQ ID NO: 4 - protein, 121 aa, synthetic construct
EVQLVESGGGLVQPGRSLRLSCAASGFTFDDYAMHWVRQAPGKGLEWVSAITNNSGHIDYADSVEGRFTISRDNAKNSLYLDMNSLRAEDTAVYYCAKVSYLSTASSLDYWGQGTLVTVSS

SEQ ID NO: 5 - protein, 121 aa, synthetic construct
EVQLVESGGGLVQPGRSLRLSCAASGFTFDDYAMHWVRQAPGKGLEWVSAITWNSGHIDYADSVEGRFTISRDNAKNSLYLDMNSLRAEDTAVYYCAKVSYLSTNSSLDYWGQGTLVTVSS

SEQ ID NO: 6 - protein, 121 aa, synthetic construct
EVQLVESGGGLVQPGRSLRLSCAASGFTFDDYAMHWVRQAPGKGLEWVSAITWNSGHIDYADSVEGRFTISRDNAKNSLYLDMNSLRAEDTAVYYCAKVSNLSTASSLDYWGQGTLVTVSS